European Patent Specification EP 3 770 177 B1, published July 8, 2026. Title: ANTI-PD-1 MONOCLONAL ANTIBODIES AND OBTAINING METHOD THEREOF. Applicant: Bejing Dongfang Biotech Co.Ltd.; Beijing Jingyitaixiang Technology Development Co.Ltd. The sequence listing filed with the application follows.

SEQUENCE LISTING (52 sequences)

SEQ ID NO: 1 - protein, 113 aa, Artificial Sequence
  The sequence is synthesized
QVQLVESGGGVVQPGRSLRLDCKASGITFSNNGMHWVRQAPGKGLEWVAVIWYDSTKKYYADSVKGRFTISRDNSKNTLFLQMNSLRAEDTAVYYCATNTDYWGQGTLVTVSS

SEQ ID NO: 2 - protein, 113 aa, Artificial Sequence
  The sequence is synthesized
QVQLVESGGGVVQPGRSLRLDCKASGITFSNYGMHWVRQAPGKGLEWVAVIWYDSSRKYYADSVKGRFTISRDNSKNTLFLQMNSLRAEDTAVYYCATNNDYWGQGTLVTVSS

SEQ ID NO: 3 - protein, 113 aa, Artificial Sequence
  The sequence is synthesized
QVQLVESGGGVVQPGRSLRLDCKASGITFSNNGMHWVRQAPGKGLEWVAVIWYDSSRKYYADSVKGRFTISRDNSKNTLFLQMNSLRAEDTAVYYCATNNDYWGQGTLVTVSS

SEQ ID NO: 4 - protein, 113 aa, Artificial Sequence
  The sequence is synthesized
QVQLVESGGGVVQPGRSLRLDCKASGITFSNYGMHWVRQAPGKGLEWVAVIWYDGSKKYYADSVKGRFTISRDNSKNTLFLQMNSLRAEDTAVYYCATNNDYWGQGTLVTVSS

SEQ ID NO: 5 - protein, 107 aa, Artificial Sequence
  The sequence is synthesized
DIQMTQSPSSLSASVGDRVTITCRASQNIHSYLDWYQQKPGKAPKLLIYEASTRASGVPSRFSGSGSGTDFTLTISSLQPEDFATYYCQQALKLPITFGQGTKVEIK

SEQ ID NO: 6 - protein, 107 aa, Artificial Sequence
  The sequence is synthesized
DIQMTQSPSSLSASVGDRVTITCRASQNVSNWLDWYQQKPGKAPKLLIYDASNRATGVPSRFSGSGSGTDFTLTISSLQPEDFATYYCQQSRHIPLTFGQGTKVEIK

SEQ ID NO: 7 - protein, 107 aa, Artificial Sequence
  The sequence is synthesized
DIQMTQSPSSLSASVGDRVTITCRASQSIHNYLDWYQQKPGKAPKLLIYNASTRATGVPSRFSGSGSGTDFTLTISSLQPEDFATYYCQQELHLPLTFGQGTKVEIK

SEQ ID NO: 8 - protein, 107 aa, Artificial Sequence
  The sequence is synthesized
DIQMTQSPSSLSASVGDRVTITCRASQDINNWLDWYQQKPGKAPKLLIYDASTLATGVPSRFSGSGSGTDFTLTISSLQPEDFATYYCQQNVNLPLTFGQGTKVEIK

SEQ ID NO: 9 - protein, 107 aa, Artificial Sequence
  The sequence is synthesized
DIQMTQSPSSLSASVGDRVTITCRASQDVRNYLDWYQQKPGKAPKLLIYGASTRATGVPSRFSGSGSGTDFTLTISSLQPEDFATYYCQQDIDLPLTFGQGTKVEIK

SEQ ID NO: 10 - protein, 107 aa, Artificial Sequence
  The sequence is synthesized
DIQMTQSPSSLSASVGDRVTITCRASQGINSWLDWYQQKPGKAPKLLIYDASTRATGVPSRFSGSGSGTDFTLTISSLQPEDFATYYCQQSYRLPLTFGQGTKVEIK

SEQ ID NO: 11 - protein, 107 aa, Artificial Sequence
  The sequence is synthesized
DIQMTQSPSSLSASVGDRVTITCRASQSVSNYLDWYQQKPGKAPKLLIYDASTRATGVPSRFSGSGSGTDFTLTISSLQPEDFATYYCQQNMQLPLTFGQGTKVEIK

SEQ ID NO: 12 - DNA, 321 bp, Artificial Sequence
  The sequence is synthesized
  misc_feature (82)..(83): r is a or g
  misc_feature (85)..(85): r is a or g
  misc_feature (88)..(88): v is a, c or g
  misc_feature (89)..(89): r is a or g
  misc_feature (92)..(92): v is a, c or g
  misc_feature (94)..(94): n is a, c, g or t
  misc_feature (95)..(95): b is c, g or t
  misc_feature (96)..(96): y is c or t
  misc_feature (100)..(100): r is a or g
  misc_feature (101)..(101): m is a or c
  misc_feature (148)..(148): r is a or g
  misc_feature (149)..(149): v is a, c or g
  misc_feature (150)..(150): k is g or t
  misc_feature (158)..(158): v is a, c or g
  misc_feature (161)..(161): k is g or t
  misc_feature (163)..(163): s is c or g
  misc_feature (164)..(164): m is a or c
  misc_feature (166)..(166): w is a or t
  misc_feature (271)..(272): n is a, c, g or t
  misc_feature (273)..(273): s is c or g
  misc_feature (274)..(275): n is a, c, g or t
  misc_feature (276)..(276): s is c or g
  misc_feature (277)..(277): v is a, c or g
  misc_feature (278)..(278): r is a or g
  misc_feature (279)..(279): b is c, g or t
  misc_feature (280)..(281): n is a, c, g or t
  misc_feature (282)..(282): s is c or g
  misc_feature (286)..(287): n is a, c, g or t
  misc_feature (288)..(288): s is c or g
gatatccagatgacccagagcccgagcagcctgagcgcgagcgtgggtgatcgcgtgaccattacctgccgcgcgagccagrrtrtcvrtavcnbyctgrmttggtatcagcagaaaccgggtaaagcgccgaaactgttaatttatrvkgccagcavcckgsmgwctggcgtgccgtcgcgttttagcggctcgggttcgggcaccgattttaccctgaccatctcgagcttgcagccggaggacttcgccacctactattgccagcaannsnnsvrbnnsccannsaccttcggtcagggcaccaaagtggagatcaaa

SEQ ID NO: 13 - DNA, 339 bp, Artificial Sequence
  The sequence is synthesized
  misc_feature (91)..(91): r is a or g
  misc_feature (92)..(92): v is a, c or g
  misc_feature (93)..(93): y is c or t
  misc_feature (97)..(97): k is g or t
  misc_feature (98)..(98): s is c or g
  misc_feature (103)..(103): m is a or c
  misc_feature (104)..(104): r is a or g
  misc_feature (105)..(105): y is c or t
  misc_feature (145)..(145): k is g or t
  misc_feature (147)..(147): m is a or c
  misc_feature (148)..(149): k is g or t
  misc_feature (150)..(150): y is c or t
  misc_feature (155)..(155): r is a or g
  misc_feature (156)..(156): n is a, c, g or t
  misc_feature (157)..(157): k is g or t
  misc_feature (158)..(158): v is a, c or g
  misc_feature (159)..(159): y is c or t
  misc_feature (160)..(161): r is a or g
  misc_feature (162)..(162): y is c or t
  misc_feature (166)..(167): r is a or g
  misc_feature (168)..(168): y is c or t
  misc_feature (169)..(169): w is a or t
  misc_feature (170)..(170): m is a or c
  misc_feature (171)..(171): y is c or t
  misc_feature (173)..(173): m is a or c
  misc_feature (174)..(174): r is a or g
  misc_feature (275)..(276): r is a or g
  misc_feature (277)..(278): v is a, c is g
  misc_feature (279)..(279): s is c or g
  misc_feature (280)..(281): n is a, c, g or t
  misc_feature (282)..(282): y is c or t
  misc_feature (283)..(284): n is a, c, g or t
  misc_feature (285)..(285): s is c or g
  misc_feature (286)..(287): n is a, c, g or t
  misc_feature (288)..(288): s is c or g
  misc_feature (289)..(290): n is a, c, g or t
  misc_feature (291)..(291): y is c or t
  misc_feature (292)..(293): n is a, c, g or t
  misc_feature (294)..(294): s is c or g
  misc_feature (295)..(296): n is a, c, g or t
  misc_feature (297)..(297): s is c or g
  misc_feature (298)..(298): h is a, c or t
  misc_feature (300)..(300): k is g or t
caggtgcagctggtggagtctgggggaggcgtggtccagcctgggaggtccctgagactcgattgtaaggcgtctggaatcaccttcagtrvytacksgatgmrytgggtccgccaggctccaggcaaggggctggagtgggtgkcmkkyattarnkvyrryggcrrywmyamrtactatgcagactccgtgaagggccgattcaccatctccagagacaattccaagaacacgctgtttctgcaaatgaacagcctgagagccgaggacacggrrvvsnnynnsnnsnnynnsnnshtkgattactggggccagggcaccctggtcaccgtctcctca

SEQ ID NO: 14 - DNA, 993 bp, Artificial Sequence
  The sequence is synthesized
gtgtcctccgcctccaccaagggcccttccgtgttccctctggccccttgctcccgctccacctccgagtccaccgccgccctgggctgcctggtgaaggactacttccctgagcctgtgaccgtgtcctggaactccggcgccctgacctccggcgtgcacaccttccctgccgtgctgcagtcctccggcctgtactccctgtcctccgtggtgaccgtgccttcctcctccctgggcaccaagacctacacctgcaacgtggaccacaagccttccaacaccaaggtggacaagcgcgtggagtccaagtacggccctccttgccctccttgccctgcccctgagttcctgggcggcccttccgtgttcctgttccctcctaagcctaaggacaccctgatgatctcccgcacccctgaggtgacctgcgtggtggtggacgtgtcccaggaggaccctgaggtgcagttcaactggtacgtggacggcgtggaggtgcacaacgccaagaccaagcctcgcgaggagcagttcaactccacctaccgcgtggtgtccgtgctgaccgtgctgcaccaggactggctgaacggcaaggagtacaagtgcaaggtgtccaacaagggcctgccttcctccatcgagaagaccatctccaaggccaagggccagcctcgcgagcctcaggtgtacaccctgcctccttcccaggaggagatgaccaagaaccaggtgtccctgacctgcctggtgaagggcttctacccttccgacatcgccgtggagtgggagtccaacggccagcctgagaacaactacaagaccacccctcctgtgctggactccgacggctccttcttcctgtactcccgcctgaccgtggacaagtcccgctggcaggagggcaacgtgttctcctgctccgtgatgcacgaggccctgcacaaccactacacccagaagtccctgtccctgtccctgggcaagtag

SEQ ID NO: 15 - protein, 330 aa, Artificial Sequence
  The sequence is synthesized
VSSASTKGPSVFPLAPCSRSTSESTAALGCLVKDYFPEPVTVSWNSGALTSGVHTFPAVLQSSGLYSLSSVVTVPSSSLGTKTYTCNVDHKPSNTKVDKRVESKYGPPCPPCPAPEFLGGPSVFLFPPKPKDTLMISRTPEVTCVVVDVSQEDPEVQFNWYVDGVEVHNAKTKPREEQFNSTYRVVSVLTVLHQDWLNGKEYKCKVSNKGLPSSIEKTISKAKGQPREPQVYTLPPSQEEMTKNQVSLTCLVKGFYPSDIAVEWESNGQPENNYKTTPPVLDSDGSFFLYSRLTVDKSRWQEGNVFSCSVMHEALHNHYTQKSLSLSLGK

SEQ ID NO: 16 - protein, 107 aa, Artificial Sequence [sequence omitted]

SEQ ID NO: 17 - DNA, 321 bp, Artificial Sequence
  The sequence is synthesized
cgtacggtggcggcgccatctgtcttcatcttcccgccatctgatgagcagttgaaatctggtaccgctagcgttgtgtgcctgctgaataacttctatcccagagaggccaaagtacagtggaaggtggataacgccctccaatcgggtaactcccaggagagtgtcacagagcaggacagcaaggacagcacctacagcctcagcagcaccctgacgctgagcaaagcagactacgagaaacacaaagtctacgcctgcgaagtcacccatcagggcctgagctcgcccgtcacaaagagcttcaacaggggagagtgt

SEQ ID NO: 18 - protein, 11 aa, Artificial Sequence
  The sequence is synthesized
RASQNIHSYLD

SEQ ID NO: 19 - protein, 11 aa, Artificial Sequence
  The sequence is synthesized
RASQNVSNWLD

SEQ ID NO: 20 - protein, 11 aa, Artificial Sequence
  The sequence is synthesized
RASQSIHNYLD

SEQ ID NO: 21 - protein, 11 aa, Artificial Sequence
  The sequence is synthesized
RASQDINNWLD

SEQ ID NO: 22 - protein, 11 aa, Artificial Sequence
  The sequence is synthesized
RASQDVRTYLD

SEQ ID NO: 23 - protein, 11 aa, Artificial Sequence
  The sequence is synthesized
RASQGINSWLD

SEQ ID NO: 24 - protein, 11 aa, Artificial Sequence
  The sequence is synthesized
RASQSVSNYLD

SEQ ID NO: 25 - protein, 7 aa, Artificial Sequence
  The sequence is synthesized
EASTRAS

SEQ ID NO: 26 - protein, 7 aa, Artificial Sequence
  The sequence is synthesized
DASNRAT

SEQ ID NO: 27 - protein, 7 aa, Artificial Sequence
  The sequence is synthesized
NASTRAT

SEQ ID NO: 28 - protein, 7 aa, Artificial Sequence
  The sequence is synthesized
DASTLAT

SEQ ID NO: 29 - protein, 7 aa, Artificial Sequence
  The sequence is synthesized
GASTRAT

SEQ ID NO: 30 - protein, 7 aa, Artificial Sequence
  The sequence is synthesized
DASTRAT

SEQ ID NO: 31 - protein, 9 aa, Artificial Sequence
  The sequence is synthesized
QQALKLPIT

SEQ ID NO: 32 - protein, 9 aa, Artificial Sequence
  The sequence is synthesized
QQSRHIPLT

SEQ ID NO: 33 - protein, 9 aa, Artificial Sequence
  The sequence is synthesized
QQELHLPLT

SEQ ID NO: 34 - protein, 9 aa, Artificial Sequence
  The sequence is synthesized
QQNVNLPLT

SEQ ID NO: 35 - protein, 9 aa, Artificial Sequence
  The sequence is synthesized
QQDIDLPLT

SEQ ID NO: 36 - protein, 9 aa, Artificial Sequence
  The sequence is synthesized
QQSYRLPLT

SEQ ID NO: 37 - protein, 9 aa, Artificial Sequence
  The sequence is synthesized
QQNMQLPLT

SEQ ID NO: 38 - protein, 6 aa, Artificial Sequence
  The sequence is synthesized
SNNGMH

SEQ ID NO: 39 - protein, 6 aa, Artificial Sequence
  The sequence is synthesized
SNYGMH

SEQ ID NO: 40 - protein, 9 aa, Artificial Sequence
  The sequence is synthesized
VIWYDGSKK

SEQ ID NO: 41 - protein, 9 aa, Artificial Sequence
  The sequence is synthesized
VIWYDSSRK

SEQ ID NO: 42 - protein, 9 aa, Artificial Sequence
  The sequence is synthesized
VIWYDSTKK

SEQ ID NO: 43 - protein, 13 aa, Artificial Sequence
  The sequence is synthesized
TAVYYCATNNDYW

SEQ ID NO: 44 - protein, 13 aa, Artificial Sequence
  The sequence is synthesized
TAVYYCATNTDYW

SEQ ID NO: 45 - DNA, 21 bp, Artificial Sequence
  The sequence is synthesized
gatatccagatgacccagagc

SEQ ID NO: 46 - DNA, 32 bp, Artificial Sequence
  The sequence is synthesized
ctaagcggccgctttgatctccactttggtgc

SEQ ID NO: 47 - DNA, 34 bp, Artificial Sequence
  The sequence is synthesized
cataccatggcccaggtgcagctggtggagtctg

SEQ ID NO: 48 - DNA, 33 bp, Artificial Sequence
  The sequence is synthesized
gctctgggtcatctggatatcggatccaccacc

SEQ ID NO: 49 - DNA, 34 bp, Artificial Sequence; identical to SEQ ID NO: 47
  The sequence is synthesized

SEQ ID NO: 50 - DNA, 27 bp, Artificial Sequence
  The sequence is synthesized
tgaggagacggtgaccagggtgccctg

SEQ ID NO: 51 - DNA, 33 bp, Artificial Sequence
  The sequence is synthesized
ctggtcaccgtctcctcaggtggtggtggtagc

SEQ ID NO: 52 - DNA, 32 bp, Artificial Sequence; identical to SEQ ID NO: 46
  The sequence is synthesized